European Patent Specification EP 3 947 682 B1, published October 11, 2023. Title: GENETICALLY-MODIFIED IMMUNE CELLS COMPRISING A MICRORNA-ADAPTED SHRNA (SHRNAMIR). Applicant: Martin, Aaron Chatterton, Jon E. Pires, Michelle. The sequence listing filed with the application follows.

SEQUENCE LISTING (123 sequences)

SEQ ID NO: 1 - DNA, 118 bp, Artificial sequence
  Synthesized
ctgtttgaatgaggcttcagtactttacagaatcgttgcctgcacatcttggaaacacttgctgggattacttcgacttcttaacccaacagaaggctcgagaaggtatattgctgtt

SEQ ID NO: 2 - DNA, 11 bp, Artificial sequence
  Synthesized
gacagtgagcg

SEQ ID NO: 3 - DNA, 19 bp, Artificial sequence
  Synthesized
tagtgaagccacagatgta

SEQ ID NO: 4 - DNA, 11 bp, Artificial sequence
  Synthesized
tgcctactgcc

SEQ ID NO: 5 - DNA, 121 bp, Artificial sequence
  Synthesized
tcggacttcaaggggctagaattcgagcaattatcttgtttactaaaactgaataccttgctatctctttgatacatttttacaaagctgaattaaaatggtataaattaaatcactttgc

SEQ ID NO: 6 - DNA, 62 bp, Artificial sequence
  Synthesized
gtaccggaggtttgaagatgccgcatttctcgagaaatgcggcatcttcaaacctttttttg

SEQ ID NO: 7 - DNA, 22 bp, Artificial sequence
  Synthesized
aaggtttgaagatgccgcattt

SEQ ID NO: 8 - DNA, 22 bp, Artificial sequence
  Synthesized
aaatgcggcatcttcaaacctc

SEQ ID NO: 9 - DNA, 22 bp, Artificial sequence
  Synthesized
cgcaaggactggtctttctata

SEQ ID NO: 10 - DNA, 22 bp, Artificial sequence
  Synthesized
tatagaaagaccagtccttgct

SEQ ID NO: 11 - DNA, 22 bp, Artificial sequence
  Synthesized
cggctatccagcgtactccaaa

SEQ ID NO: 12 - DNA, 22 bp, Artificial sequence
  Synthesized
tttggagtacgctggatagcct

SEQ ID NO: 13 - DNA, 22 bp, Artificial sequence
  Synthesized
cgcagagaatggaaagtcaaat

SEQ ID NO: 14 - DNA, 22 bp, Artificial sequence
  Synthesized
atttgactttccattctctgct

SEQ ID NO: 15 - DNA, 22 bp, Artificial sequence
  Synthesized
cgcttatacacttacactttat

SEQ ID NO: 16 - DNA, 22 bp, Artificial sequence
  Synthesized
ataaagtgtaagtgtataagca

SEQ ID NO: 17 - DNA, 22 bp, Artificial sequence
  Synthesized
cggacatgatcttctttataat

SEQ ID NO: 18 - DNA, 22 bp, Artificial sequence
  Synthesized
attataaagaagatcatgtcca

SEQ ID NO: 19 - DNA, 22 bp, Artificial sequence
  Synthesized
acgtgcataagttaacttccaa

SEQ ID NO: 20 - DNA, 22 bp, Artificial sequence
  Synthesized
ttggaagttaacttatgcacgc

SEQ ID NO: 21 - DNA, 22 bp, Artificial sequence
  Synthesized
ctgtattaattggctctataaa

SEQ ID NO: 22 - DNA, 22 bp, Artificial sequence
  Synthesized
tttatagagccaattaatacat

SEQ ID NO: 23 - DNA, 22 bp, Artificial sequence
  Synthesized
acatgtttggcagatactataa

SEQ ID NO: 24 - DNA, 22 bp, Artificial sequence
  Synthesized
ttatagtatctgccaaacatgg

SEQ ID NO: 25 - DNA, 22 bp, Artificial sequence
  Synthesized
agagtctgaagtcacattgtaa

SEQ ID NO: 26 - DNA, 22 bp, Artificial sequence
  Synthesized
ttacaatgtgacttcagactcg

SEQ ID NO: 27 - DNA, 22 bp, Artificial sequence
  Synthesized
ggacctcaagagctccaatatc

SEQ ID NO: 28 - DNA, 22 bp, Artificial sequence
  Synthesized
gatattggagctcttgaggtct

SEQ ID NO: 29 - DNA, 22 bp, Artificial sequence
  Synthesized
agacctcaagagctccaatatc

SEQ ID NO: 30 - DNA, 22 bp, Artificial sequence
  Synthesized
gatattggagctcttgaggtcc

SEQ ID NO: 31 - DNA, 22 bp, Artificial sequence
  Synthesized
ccctgacttgttgctagtcata

SEQ ID NO: 32 - DNA, 22 bp, Artificial sequence
  Synthesized
tatgactagcaacaagtcagga

SEQ ID NO: 33 - DNA, 22 bp, Artificial sequence
  Synthesized
agcagtcaagatctttccctat

SEQ ID NO: 34 - DNA, 22 bp, Artificial sequence
  Synthesized
atagggaaagatcttgactgcc

SEQ ID NO: 35 - DNA, 22 bp, Artificial sequence
  Synthesized
agcacgttcagaagtcggttaa

SEQ ID NO: 36 - DNA, 22 bp, Artificial sequence
  Synthesized
ttaaccgacttctgaacgtgcg

SEQ ID NO: 37 - DNA, 22 bp, Artificial sequence
  Synthesized
accaccatcactcgcaagagaa

SEQ ID NO: 38 - DNA, 22 bp, Artificial sequence
  Synthesized
ttctcttgcgagtgatggtggc

SEQ ID NO: 39 - DNA, 22 bp, Artificial sequence
  Synthesized
acctcctggttatggtacagat

SEQ ID NO: 40 - DNA, 22 bp, Artificial sequence
  Synthesized
atctgtaccataaccaggaggc

SEQ ID NO: 41 - DNA, 324 bp, Artificial sequence
  Synthesized
ctgtttgaatgaggcttcagtactttacagaatcgttgcctgcacatcttggaaacacttgctgggattacttcgacttcttaacccaacagaaggctcgagaaggtatattgctgttgacagtgagcgaaggtttgaagatgccgcattttagtgaagccacagatgtaaaatgcggcatcttcaaacctctgcctactgcctcggacttcaaggggctagaattcgagcaattatcttgtttactaaaactgaataccttgctatctctttgatacatttttacaaagctgaattaaaatggtataaattaaatcactttgc

SEQ ID NO: 42 - DNA, 324 bp, Artificial sequence
  Synthesized
ctgtttgaatgaggcttcagtactttacagaatcgttgcctgcacatcttggaaacacttgctgggattacttcgacttcttaacccaacagaaggctcgagaaggtatattgctgttgacagtgagcgcgcaaggactggtctttctatatagtgaagccacagatgtatatagaaagaccagtccttgcttgcctactgcctcggacttcaaggggctagaattcgagcaattatcttgtttactaaaactgaataccttgctatctctttgatacatttttacaaagctgaattaaaatggtataaattaaatcactttgc

SEQ ID NO: 43 - DNA, 324 bp, Artificial sequence
  Synthesized
ctgtttgaatgaggcttcagtactttacagaatcgttgcctgcacatcttggaaacacttgctgggattacttcgacttcttaacccaacagaaggctcgagaaggtatattgctgttgacagtgagcgcggctatccagcgtactccaaatagtgaagccacagatgtatttggagtacgctggatagccttgcctactgcctcggacttcaaggggctagaattcgagcaattatcttgtttactaaaactgaataccttgctatctctttgatacatttttacaaagctgaattaaaatggtataaattaaatcactttgc

SEQ ID NO: 44 - DNA, 324 bp, Artificial sequence
  Synthesized
ctgtttgaatgaggcttcagtactttacagaatcgttgcctgcacatcttggaaacacttgctgggattacttcgacttcttaacccaacagaaggctcgagaaggtatattgctgttgacagtgagcgcgcagagaatggaaagtcaaattagtgaagccacagatgtaatttgactttccattctctgcttgcctactgcctcggacttcaaggggctagaattcgagcaattatcttgtttactaaaactgaataccttgctatctctttgatacatttttacaaagctgaattaaaatggtataaattaaatcactttgc

SEQ ID NO: 45 - DNA, 324 bp, Artificial sequence
  Synthesized
ctgtttgaatgaggcttcagtactttacagaatcgttgcctgcacatcttggaaacacttgctgggattacttcgacttcttaacccaacagaaggctcgagaaggtatattgctgttgacagtgagcgcgcttatacacttacactttattagtgaagccacagatgtaataaagtgtaagtgtataagcatgcctactgcctcggacttcaaggggctagaattcgagcaattatcttgtttactaaaactgaataccttgctatctctttgatacatttttacaaagctgaattaaaatggtataaattaaatcactttgc

SEQ ID NO: 46 - DNA, 324 bp, Artificial sequence
  Synthesized
ctgtttgaatgaggcttcagtactttacagaatcgttgcctgcacatcttggaaacacttgctgggattacttcgacttcttaacccaacagaaggctcgagaaggtatattgctgttgacagtgagcgcggacatgatcttctttataattagtgaagccacagatgtaattataaagaagatcatgtccatgcctactgcctcggacttcaaggggctagaattcgagcaattatcttgtttactaaaactgaataccttgctatctctttgatacatttttacaaagctgaattaaaatggtataaattaaatcactttgc

SEQ ID NO: 47 - DNA, 324 bp, Artificial sequence
  Synthesized
ctgtttgaatgaggcttcagtactttacagaatcgttgcctgcacatcttggaaacacttgctgggattacttcgacttcttaacccaacagaaggctcgagaaggtatattgctgttgacagtgagcgacgtgcataagttaacttccaatagtgaagccacagatgtattggaagttaacttatgcacgctgcctactgcctcggacttcaaggggctagaattcgagcaattatcttgtttactaaaactgaataccttgctatctctttgatacatttttacaaagctgaattaaaatggtataaattaaatcactttgc

SEQ ID NO: 48 - DNA, 324 bp, Artificial sequence
  Synthesized
ctgtttgaatgaggcttcagtactttacagaatcgttgcctgcacatcttggaaacacttgctgggattacttcgacttcttaacccaacagaaggctcgagaaggtatattgctgttgacagtgagcgctgtattaattggctctataaatagtgaagccacagatgtatttatagagccaattaatacattgcctactgcctcggacttcaaggggctagaattcgagcaattatcttgtttactaaaactgaataccttgctatctctttgatacatttttacaaagctgaattaaaatggtataaattaaatcactttgc

SEQ ID NO: 49 - DNA, 324 bp, Artificial sequence
  Synthesized
ctgtttgaatgaggcttcagtactttacagaatcgttgcctgcacatcttggaaacacttgctgggattacttcgacttcttaacccaacagaaggctcgagaaggtatattgctgttgacagtgagcgacatgtttggcagatactataatagtgaagccacagatgtattatagtatctgccaaacatggtgcctactgcctcggacttcaaggggctagaattcgagcaattatcttgtttactaaaactgaataccttgctatctctttgatacatttttacaaagctgaattaaaatggtataaattaaatcactttgc

SEQ ID NO: 50 - DNA, 324 bp, Artificial sequence
  Synthesized
ctgtttgaatgaggcttcagtactttacagaatcgttgcctgcacatcttggaaacacttgctgggattacttcgacttcttaacccaacagaaggctcgagaaggtatattgctgttgacagtgagcgagagtctgaagtcacattgtaatagtgaagccacagatgtattacaatgtgacttcagactcgtgcctactgcctcggacttcaaggggctagaattcgagcaattatcttgtttactaaaactgaataccttgctatctctttgatacatttttacaaagctgaattaaaatggtataaattaaatcactttgc

SEQ ID NO: 51 - DNA, 322 bp, Artificial sequence
  Synthesized
ctgtttgaatgaggcttcagtactttacagaatcgttgcctgcacatcttggaaacacttgctgggattacttcgacttcttaacccaacagaaggctcgagaaggtatattgctgttgacagtgagcggacctcaagagctccaatatctagtgaagccacagatgtagatattggagctcttgaggtctgcctactgcctcggacttcaaggggctagaattcgagcaattatcttgtttactaaaactgaataccttgctatctctttgatacatttttacaaagctgaattaaaatggtataaattaaatcactttgc

SEQ ID NO: 52 - DNA, 324 bp, Artificial sequence
  Synthesized
ctgtttgaatgaggcttcagtactttacagaatcgttgcctgcacatcttggaaacacttgctgggattacttcgacttcttaacccaacagaaggctcgagaaggtatattgctgttgacagtgagcgagacctcaagagctccaatatctagtgaagccacagatgtagatattggagctcttgaggtcctgcctactgcctcggacttcaaggggctagaattcgagcaattatcttgtttactaaaactgaataccttgctatctctttgatacatttttacaaagctgaattaaaatggtataaattaaatcactttgc

SEQ ID NO: 53 - DNA, 324 bp, Artificial sequence
  Synthesized
ctgtttgaatgaggcttcagtactttacagaatcgttgcctgcacatcttggaaacacttgctgggattacttcgacttcttaacccaacagaaggctcgagaaggtatattgctgttgacagtgagcgccctgacttgttgctagtcatatagtgaagccacagatgtatatgactagcaacaagtcaggatgcctactgcctcggacttcaaggggctagaattcgagcaattatcttgtttactaaaactgaataccttgctatctctttgatacatttttacaaagctgaattaaaatggtataaattaaatcactttgc

SEQ ID NO: 54 - DNA, 324 bp, Artificial sequence
  Synthesized
ctgtttgaatgaggcttcagtactttacagaatcgttgcctgcacatcttggaaacacttgctgggattacttcgacttcttaacccaacagaaggctcgagaaggtatattgctgttgacagtgagcgagcagtcaagatctttccctattagtgaagccacagatgtaatagggaaagatcttgactgcctgcctactgcctcggacttcaaggggctagaattcgagcaattatcttgtttactaaaactgaataccttgctatctctttgatacatttttacaaagctgaattaaaatggtataaattaaatcactttgc

SEQ ID NO: 55 - DNA, 324 bp, Artificial sequence
  Synthesized
ctgtttgaatgaggcttcagtactttacagaatcgttgcctgcacatcttggaaacacttgctgggattacttcgacttcttaacccaacagaaggctcgagaaggtatattgctgttgacagtgagcgagcacgttcagaagtcggttaatagtgaagccacagatgtattaaccgacttctgaacgtgcgtgcctactgcctcggacttcaaggggctagaattcgagcaattatcttgtttactaaaactgaataccttgctatctctttgatacatttttacaaagctgaattaaaatggtataaattaaatcactttgc

SEQ ID NO: 56 - DNA, 324 bp, Artificial sequence
  Synthesized
ctgtttgaatgaggcttcagtactttacagaatcgttgcctgcacatcttggaaacacttgctgggattacttcgacttcttaacccaacagaaggctcgagaaggtatattgctgttgacagtgagcgaccaccatcactcgcaagagaatagtgaagccacagatgtattctcttgcgagtgatggtggctgcctactgcctcggacttcaaggggctagaattcgagcaattatcttgtttactaaaactgaataccttgctatctctttgatacatttttacaaagctgaattaaaatggtataaattaaatcactttgc

SEQ ID NO: 57 - DNA, 324 bp, Artificial sequence
  Synthesized
ctgtttgaatgaggcttcagtactttacagaatcgttgcctgcacatcttggaaacacttgctgggattacttcgacttcttaacccaacagaaggctcgagaaggtatattgctgttgacagtgagcgacctcctggttatggtacagattagtgaagccacagatgtaatctgtaccataaccaggaggctgcctactgcctcggacttcaaggggctagaattcgagcaattatcttgtttactaaaactgaataccttgctatctctttgatacatttttacaaagctgaattaaaatggtataaattaaatcactttgc

SEQ ID NO: 58 - DNA, 22 bp, Homo sapiens
tggcctggagcaacaaatctga

SEQ ID NO: 59 - DNA, 22 bp, Homo sapiens
accggacctcgttgtttagact

SEQ ID NO: 60 - DNA, 22 bp, Homo sapiens
ctatctcttgtactacactgaa

SEQ ID NO: 61 - DNA, 22 bp, Homo sapiens
gatagagaacatgatgtgactt

SEQ ID NO: 62 - DNA, 22 bp, Homo sapiens
cccgggggattgctcacctcca

SEQ ID NO: 63 - DNA, 22 bp, Homo sapiens
gggccccctaacgagtggaggt

SEQ ID NO: 64 - protein, 354 aa, Artificial sequence
  Synthesized
MNTKYNKEFLLYLAGFVDGDGSIYACIEPDQSRKFKHTLRLYFEVGQKTQRRWFLDKLVDEIGVGYVYDRGSVSNYRLSEIKPLHNFLTQLQPFLKLKQKQANLVLKIIEQLPSAKESPDKFLEVCTWVDQIAALNDSKTRKTTSETVRAVLDSLPGSVGGLSPSQASSAASSASSSPGSGISEALRAGAGSGTGYNKEFLLYLAGFVDGDGSIFACITPSQTHKFKHRLFLRFTVGQKTQRRWFLDKLVDEIGVGYVVDSGSVSEYRLSQIKPLHNFLTQLQPFLKLKQKQANLVLKIIEQLPSAKESPDKFLEVCTWVDQIAALNDSKTRKTTSETVRAVLDSLSEKKKSSP

SEQ ID NO: 65 - protein, 354 aa, Artificial sequence
  Synthesized
MNTKYNKEFLLYLAGFVDGDGSIYACITPKQRSKFKHSLRLRFTVGQKTQRRWFLDKLVDEIGVGYVLDGGGVSEYRLSEIKPLHNFLTQLQPFLKLKQKQANLVLKIIEQLPSAKESPDKFLEVCTWVDQIAALNDSKTRKTTSETVRAVLDSLPGSVGGLSPSQASSATSSASSSPGSGISEALRAGAGSGTGYNKEFLLYLAGFVDGDGSIYACIEPDQSRKFKHTLRLYFEVGQKTQRRWFLDKLVDEIGVGYVYDRGSVSNYRLSEIKPLHNFLTQLQPFLKLKQKQANLVLKIIEQLPSAKESPDKFLEVCTWVDQIAALNDSKTRKTTSETVRAVLDSLSEKKKSSP

SEQ ID NO: 66 - protein, 325 aa, Artificial sequence
  Synthesized
VMAPRTLFLGGGGSGGGGSGGGGSIQRTPKIQVYSRHPAENGKSNFLNCYVSGFHPSDIEVDLLKNGERIEKVEHSDLSFSKDWSFYLLYYTEFTPTEKDEYACRVNHVTLSQPKIVKWDRDMGGGGSGGGGSGGGGSGGGGSGSHSLKYFHTSVSRPGRGEPRFISVGYVDDTQFVRFDNDAASPRMVPRAPWMEQEGSEYWDRETRSARDTAQIFRVNLRTLRGYYNQSEAGSHTLQWMHGCELGPDGRFLRGYEQFAYDGKDYLTLNEDLRSWTAVDTAAQISEQKSNDASEAEHQRAYLEDTCVEWLHKYLEKGKETLLHL

SEQ ID NO: 67 - DNA, 164 bp, Artificial sequence
  Synthesized
gggcggagttagggcggagccaatcagcgtgcgccgttccgaaagttgccttttatggctgggcggagaatgggcggtgaacgccgatgattatataaggacgcgccgggtgtggcacagctagttccgtcgcagccgggatttgggtcgcggttcttgtttgt

SEQ ID NO: 68 - DNA, 207 bp, Artificial sequence
  Synthesized
gatccagacatgataagatacattgatgagtttggacaaaccacaactagaatgcagtgaaaaaaatgctttatttgtgaaatttgtgatgctattgctttatttgtaaccattataagctgcaataaacaagttaacaacaacaattgcattcattttatgtttcaggttcagggggaggtgtgggaggttttttaaagcaagtaa

SEQ ID NO: 69 - DNA, 133 bp, Artificial sequence
  Synthesized
gtaagtattaatgttacaagacaggtttaaggacaccaatagaaactgggcttgtcgagacagagaagactcttgcgtttctgataggcacctattggtcttactgacatccactttgcctttctctccacag

SEQ ID NO: 70 - DNA, 81 bp, Artificial sequence
  Synthesized
cgggccaagagatctggaagcggcgccacaaatttctcactgctgaaacaggccggcgacgtggaagagaaccctggacct

SEQ ID NO: 71 - DNA, 225 bp, Artificial sequence
  Synthesized
ctgtgccttctagttgccagccatctgttgtttgcccctcccccgtgccttccttgaccctggaaggtgccactcccactgtcctttcctaataaaatgaggaaattgcatcgcattgtctgagtaggtgtcattctattctggggggtggggtggggcaggacagcaagggggaggattgggaagacaatagcaggcatgctggggatgcggtgggctctatgg

SEQ ID NO: 72 - DNA, 212 bp, Artificial sequence
  Synthesized
gggcagagcgcacatcgcccacagtccccgagaagttggggggaggggtcggcaattgaacgggtgcctagagaaggtggcgcggggtaaactgggaaagtgatgtcgtgtactggctccgcctttttcccgagggtgggggagaaccgtatataagtgcagtagtcgccgtgaacgttctttttcgcaacgggtttgccgccagaacacag

SEQ ID NO: 73 - protein, 20 aa, Artificial sequence
  Synthesized
MEAPAQLLFLLLLWLPSSRA

SEQ ID NO: 74 - DNA, 3885 bp, Artificial sequence
  Synthesized
gggcggagttagggcggagccaatcagcgtgcgccgttccgaaagttgccttttatggctgggcggagaatgggcggtgaacgccgatgattatataaggacgcgccgggtgtggcacagctagttccgtcgcagccgggatttgggtcgcggttcttgtttgtgccaccatggaggctcctgctcagctgctgttcctgctcctgctgtggctgcccagcagcagagctgacatacagatgactcagactacctcttccctatctgcttctttaggcgaccgagtaacaatatcttgccgggccagccaggacatctcaaaatacttaaactggtatcagcagaagccggacggaacagttaagttgctcatttaccacacgtcgagattacactcaggcgttcctagccgattttcgggttccggttccggtacggactacagcctgacaatcagtaaccttgagcaggaggacatcgccacctacttctgtcagcagggcaacacgctcccgtacacattcggtgggggaactaagctggagattaccggaggcggtggcagcggtggcggcggcagcgggggtggcggctcggaggtcaagttacaggagagcggaccgggcttggtcgcacctagccagagcctctcagtcacgtgcactgtgtctggagtcagtctcccagactacggggtatcatggatacgacagccgcctagaaagggcttagagtggctgggggttatctggggaagtgaaaccacatactacaactcagctctcaagagccgcctcaccatcattaaggacaacagtaagtcgcaggttttcttaaagatgaactctctccagactgacgacaccgctatttactactgcgcgaagcactactactacggcgggagttacgcaatggactactggggtcagggcacttctgtgaccgtatccagcactactaccccagccccacgtccccccacgccagctccaacgatagcaagtcagcccttatctcttcgccctgaggcttgcaggcccgcggcgggcggcgccgttcacacgcgaggactagacttcgcctgcgacatctacatctgggcaccactagccgggacttgcggagtgttgttgttgagcttggtaataacgctctactgcaaagcgagccgcaaaaaagcggcggcggcggcgaaaagcccgtttgcgagcccggcgagcagcgcgcaggaagaagatgcgagcagctgccgcgcgccgagcgaagaagaaggcagctgcgaactgagagtgaagttctctcgctccgcggacgcacccgcttaccagcagggtcagaaccagctatacaacgagttaaacctggggcgccgggaggagtacgacgtgttagacaagcgtagaggtagggacccggagatgggaggcaagcctcggagaaagaacccccaggagggcctgtacaacgaactccagaaggacaagatggctgaggcgtactcggagattggtatgaagggcgagagacgtcgcggaaagggacacgacggcttataccaggggctttccaccgcgaccaaggacacatacgacgcgctgcacatgcaagccttaccacctcgacgggccaagagatctggaagcggcgccacaaatttctcactgctgaaacaggccggcgacgtggaagagaaccctggacctatgtctcgctccgtggccttagctgtgctcgcgctactctctctttctggcctggaggctgtgatggcgccgcgcaccctgtttctgggaggcgggggtagcggtgggggcggaagcgggggaggcggcagcatccagcgtactccaaagattcaggtttactcacgtcatccagcagagaatggaaagtcaaatttcctgaattgctatgtgtctgggtttcatccatccgacattgaagttgacttactgaagaatggagagagaattgaaaaagtggagcattcagacttgtctttcagcaaggactggtctttctacctgctctattatacggaattcacccccactgaaaaagatgagtatgcctgccgtgtgaaccatgtgactttgtcacagcccaagatagttaagtgggatcgagacatgggcggtggcggtagcggaggtggaggtagcggtggtggaggcagcggtggaggcggcagcggctcccactccttgaagtatttccacacttccgtgtcccggcccggccgcggggagccccgcttcatctctgtgggctacgtggacgacacccagttcgtgcgcttcgacaacgacgccgcgagtccgaggatggtgccgcgggcgccgtggatggagcaggaggggtcagagtattgggaccgggagacacggagcgccagggacaccgcacagattttccgagtgaatctgcggacgctgcgcggctactacaatcagagcgaggccggctctcacaccctgcagtggatgcatggctgcgagctggggcccgacgggcgcttcctccgcgggtatgaacagttcgcctacgacggcaaggattatctcaccctgaatgaggacctgcgctcctggaccgcggtggacacggcggctcagatctccgagcaaaagtcaaatgatgcctctgaggcggagcaccagagagcctacctggaagacacatgcgtggagtggctccacaaatacctggagaaggggaaggagacgctgcttcacctgggtaagtattaatgttacaagacaggtttaaggacaccaatagaaactgggcttgtcgagacagagagtacctgtttgaatgaggcttcagtactttacagaatcgttgcctgcacatcttggaaacacttgctgggattacttcgacttcttaacccaacagaaggctcgagaaggtatattgctgttgacagtgagcgcggacatgatcttctttataattagtgaagccacagatgtaattataaagaagatcatgtccatgcctactgcctcggacttcaaggggctagaattcgagcaattatcttgtttactaaaactgaataccttgctatctctttgatacatttttacaaagctgaattaaaatggtataaattaaatcactttgcggccagactcttgcgtttctgataggcacctattggtcttactgacatccactttgcctttctctccacagagcccccaaagacacacgtgactcaccaccccatctctgaccatgaggccaccctgaggtgctgggccctgggcttctaccctgcggagatcacactgacctggcagcaggatggggagggccatacccaggacacggagctcgtggaaaccaggcctgcaggggatggaaccttccagaagtgggcagctgtggtggtgccttctggagaggagcagagatacacgtgccatgtgcagcatgaggggctacccgagcccgtcaccctgagatggaagccggcttcccagcccaccatccccatcgtgggcatcattgctggcctggttctccttggatctgtggtatctggagctgtggttgctgctgtgatatggaggaagaagagctcaggtggaaaaggagggagctactctaaggctgagtggagcgacagtgcccaggggtctgagtctcacagcttgtaaggtagatccagacatgataagatacattgatgagtttggacaaaccacaactagaatgcagtgaaaaaaatgctttatttgtgaaatttgtgatgctattgctttatttgtaaccattataagctgcaataaacaagttaacaacaacaattgcattcattttatgtttcaggttcagggggaggtgtgggaggttttttaaagcaagtaa

SEQ ID NO: 75 - DNA, 4262 bp, Artificial sequence
  Synthesized
gggcggagttagggcggagccaatcagcgtgcgccgttccgaaagttgccttttatggctgggcggagaatgggcggtgaacgccgatgattatataaggacgcgccgggtgtggcacagctagttccgtcgcagccgggatttgggtcgcggttcttgtttgtgccaccatggaggctcctgctcagctgctgttcctgctcctgctgtggctgcccagcagcagagctgacatacagatgactcagactacctcttccctatctgcttctttaggcgaccgagtaacaatatcttgccgggccagccaggacatctcaaaatacttaaactggtatcagcagaagccggacggaacagttaagttgctcatttaccacacgtcgagattacactcaggcgttcctagccgattttcgggttccggttccggtacggactacagcctgacaatcagtaaccttgagcaggaggacatcgccacctacttctgtcagcagggcaacacgctcccgtacacattcggtgggggaactaagctggagattaccggaggcggtggcagcggtggcggcggcagcgggggtggcggctcggaggtcaagttacaggagagcggaccgggcttggtcgcacctagccagagcctctcagtcacgtgcactgtgtctggagtcagtctcccagactacggggtatcatggatacgacagccgcctagaaagggcttagagtggctgggggttatctggggaagtgaaaccacatactacaactcagctctcaagagccgcctcaccatcattaaggacaacagtaagtcgcaggttttcttaaagatgaactctctccagactgacgacaccgctatttactactgcgcgaagcactactactacggcgggagttacgcaatggactactggggtcagggcacttctgtgaccgtatccagcactactaccccagccccacgtccccccacgccagctccaacgatagcaagtcagcccttatctcttcgccctgaggcttgcaggcccgcggcgggcggcgccgttcacacgcgaggactagacttcgcctgcgacatctacatctgggcaccactagccgggacttgcggagtgttgttgttgagcttggtaataacgctctactgcaaagcgagccgcaaaaaagcggcggcggcggcgaaaagcccgtttgcgagcccggcgagcagcgcgcaggaagaagatgcgagcagctgccgcgcgccgagcgaagaagaaggcagctgcgaactgagagtgaagttctctcgctccgcggacgcacccgcttaccagcagggtcagaaccagctatacaacgagttaaacctggggcgccgggaggagtacgacgtgttagacaagcgtagaggtagggacccggagatgggaggcaagcctcggagaaagaacccccaggagggcctgtacaacgaactccagaaggacaagatggctgaggcgtactcggagattggtatgaagggcgagagacgtcgcggaaagggacacgacggcttataccaggggctttccaccgcgaccaaggacacatacgacgcgctgcacatgcaagccttaccacctcgatgaagccgatccagacatgataagatacattgatgagtttggacaaaccacaactagaatgcagtgaaaaaaatgctttatttgtgaaatttgtgatgctattgctttatttgtaaccattataagctgcaataaacaagttaacaacaacaattgcattcattttatgtttcaggttcagggggaggtgtgggaggttttttaaagcaagtaattcggggcagagcgcacatcgcccacagtccccgagaagttggggggaggggtcggcaattgaacgggtgcctagagaaggtggcgcggggtaaactgggaaagtgatgtcgtgtactggctccgcctttttcccgagggtgggggagaaccgtatataagtgcagtagtcgccgtgaacgttctttttcgcaacgggtttgccgccagaacacagccatgccaccatgtctcgctccgtggccttagctgtgctcgcgctactctctctttctggcctggaggctgtgatggcgccgcgcaccctgtttctgggaggcgggggtagcggtgggggcggaagcgggggaggcggcagcatccagcgtactccaaagattcaggtttactcacgtcatccagcagagaatggaaagtcaaatttcctgaattgctatgtgtctgggtttcatccatccgacattgaagttgacttactgaagaatggagagagaattgaaaaagtggagcattcagacttgtctttcagcaaggactggtctttctacctgctctattatacggaattcacccccactgaaaaagatgagtatgcctgccgtgtgaaccatgtgactttgtcacagcccaagatagttaagtgggatcgagacatgggcggtggcggtagcggaggtggaggtagcggtggtggaggcagcggtggaggcggcagcggctcccactccttgaagtatttccacacttccgtgtcccggcccggccgcggggagccccgcttcatctctgtgggctacgtggacgacacccagttcgtgcgcttcgacaacgacgccgcgagtccgaggatggtgccgcgggcgccgtggatggagcaggaggggtcagagtattgggaccgggagacacggagcgccagggacaccgcacagattttccgagtgaatctgcggacgctgcgcggctactacaatcagagcgaggccggctctcacaccctgcagtggatgcatggctgcgagctggggcccgacgggcgcttcctccgcgggtatgaacagttcgcctacgacggcaaggattatctcaccctgaatgaggacctgcgctcctggaccgcggtggacacggcggctcagatctccgagcaaaagtcaaatgatgcctctgaggcggagcaccagagagcctacctggaagacacatgcgtggagtggctccacaaatacctggagaaggggaaggagacgctgcttcacctgggtaagtattaatgttacaagacaggtttaaggacaccaatagaaactgggcttgtcgagacagagagtacctgtttgaatgaggcttcagtactttacagaatcgttgcctgcacatcttggaaacacttgctgggattacttcgacttcttaacccaacagaaggctcgagaaggtatattgctgttgacagtgagcgcggacatgatcttctttataattagtgaagccacagatgtaattataaagaagatcatgtccatgcctactgcctcggacttcaaggggctagaattcgagcaattatcttgtttactaaaactgaataccttgctatctctttgatacatttttacaaagctgaattaaaatggtataaattaaatcactttgcggccagactcttgcgtttctgataggcacctattggtcttactgacatccactttgcctttctctccacagagcccccaaagacacacgtgactcaccaccccatctctgaccatgaggccaccctgaggtgctgggccctgggcttctaccctgcggagatcacactgacctggcagcaggatggggagggccatacccaggacacggagctcgtggaaaccaggcctgcaggggatggaaccttccagaagtgggcagctgtggtggtgccttctggagaggagcagagatacacgtgccatgtgcagcatgaggggctacccgagcccgtcaccctgagatggaagccggcttcccagcccaccatccccatcgtgggcatcattgctggcctggttctccttggatctgtggtatctggagctgtggttgctgctgtgatatggaggaagaagagctcaggtggaaaaggagggagctactctaaggctgagtggagcgacagtgcccaggggtctgagtctcacagcttgtaaatggctgtgccttctagttgccagccatctgttgtttgcccctcccccgtgccttccttgaccctggaaggtgccactcccactgtcctttcctaataaaatgaggaaattgcatcgcattgtctgagtaggtgtcattctattctggggggtggggtggggcaggacagcaagggggaggattgggaagacaatagcaggcatgctggggatgcggtgggctctatgg

SEQ ID NO: 76 - DNA, 22 bp, Artificial sequence
  Synthesized
cgcaaggcattcctcttgaata

SEQ ID NO: 77 - DNA, 22 bp, Artificial sequence
  Synthesized
tattcaagaggaatgccttgct

SEQ ID NO: 78 - DNA, 22 bp, Artificial sequence
  Synthesized
cggcattcctcttgaatattta

SEQ ID NO: 79 - DNA, 22 bp, Artificial sequence
  Synthesized
taaatattcaagaggaatgcct

SEQ ID NO: 80 - DNA, 22 bp, Artificial sequence
  Synthesized
cggtttcttattcaaagatgat

SEQ ID NO: 81 - DNA, 22 bp, Artificial sequence
  Synthesized
atcatctttgaataagaaacca

SEQ ID NO: 82 - DNA, 22 bp, Artificial sequence
  Synthesized
agctcctgcataggacactgaa

SEQ ID NO: 83 - DNA, 22 bp, Artificial sequence
  Synthesized
ttcagtgtcctatgcaggagcc

SEQ ID NO: 84 - DNA, 22 bp, Artificial sequence
  Synthesized
cggctagaaagcatccattaat

SEQ ID NO: 85 - DNA, 22 bp, Artificial sequence
  Synthesized
attaatggatgctttctagcct

SEQ ID NO: 86 - DNA, 324 bp, Artificial sequence
  Synthesized
ctgtttgaatgaggcttcagtactttacagaatcgttgcctgcacatcttggaaacacttgctgggattacttcgacttcttaacccaacagaaggctcgagaaggtatattgctgttgacagtgagcgcgcaaggcattcctcttgaatatagtgaagccacagatgtatattcaagaggaatgccttgcttgcctactgcctcggacttcaaggggctagaattcgagcaattatcttgtttactaaaactgaataccttgctatctctttgatacatttttacaaagctgaattaaaatggtataaattaaatcactttgc

SEQ ID NO: 87 - DNA, 324 bp, Artificial sequence
  Synthesized
ctgtttgaatgaggcttcagtactttacagaatcgttgcctgcacatcttggaaacacttgctgggattacttcgacttcttaacccaacagaaggctcgagaaggtatattgctgttgacagtgagcgcggcattcctcttgaatatttatagtgaagccacagatgtataaatattcaagaggaatgccttgcctactgcctcggacttcaaggggctagaattcgagcaattatcttgtttactaaaactgaataccttgctatctctttgatacatttttacaaagctgaattaaaatggtataaattaaatcactttgc

SEQ ID NO: 88 - DNA, 324 bp, Artificial sequence
  Synthesized
ctgtttgaatgaggcttcagtactttacagaatcgttgcctgcacatcttggaaacacttgctgggattacttcgacttcttaacccaacagaaggctcgagaaggtatattgctgttgacagtgagcgcggtttcttattcaaagatgattagtgaagccacagatgtaatcatctttgaataagaaaccatgcctactgcctcggacttcaaggggctagaattcgagcaattatcttgtttactaaaactgaataccttgctatctctttgatacatttttacaaagctgaattaaaatggtataaattaaatcactttgc

SEQ ID NO: 89 - DNA, 324 bp, Artificial sequence
  Synthesized
ctgtttgaatgaggcttcagtactttacagaatcgttgcctgcacatcttggaaacacttgctgggattacttcgacttcttaacccaacagaaggctcgagaaggtatattgctgttgacagtgagcgagctcctgcataggacactgaatagtgaagccacagatgtattcagtgtcctatgcaggagcctgcctactgcctcggacttcaaggggctagaattcgagcaattatcttgtttactaaaactgaataccttgctatctctttgatacatttttacaaagctgaattaaaatggtataaattaaatcactttgc

SEQ ID NO: 90 - DNA, 324 bp, Artificial sequence
  Synthesized
ctgtttgaatgaggcttcagtactttacagaatcgttgcctgcacatcttggaaacacttgctgggattacttcgacttcttaacccaacagaaggctcgagaaggtatattgctgttgacagtgagcgcggctagaaagcatccattaattagtgaagccacagatgtaattaatggatgctttctagccttgcctactgcctcggacttcaaggggctagaattcgagcaattatcttgtttactaaaactgaataccttgctatctctttgatacatttttacaaagctgaattaaaatggtataaattaaatcactttgc

SEQ ID NO: 91 - DNA, 22 bp, Artificial sequence
  Synthesized
aagatgtgatggacttctataa

SEQ ID NO: 92 - DNA, 22 bp, Artificial sequence
  Synthesized
ttatagaagtccatcacatctc

SEQ ID NO: 93 - DNA, 22 bp, Artificial sequence
  Synthesized
aaccaacggtggcaatgtgaaa

SEQ ID NO: 94 - DNA, 22 bp, Artificial sequence
  Synthesized
tttcacattgccaccgttggtg

SEQ ID NO: 95 - DNA, 22 bp, Artificial sequence
  Synthesized
aggtggcaatgtgaaattgtat

SEQ ID NO: 96 - DNA, 22 bp, Artificial sequence
  Synthesized
atacaatttcacattgccaccg

SEQ ID NO: 97 - DNA, 22 bp, Artificial sequence
  Synthesized
agcaagctttcctggagcaaat

SEQ ID NO: 98 - DNA, 22 bp, Artificial sequence
  Synthesized
atttgctccaggaaagcttgcc

SEQ ID NO: 99 - DNA, 22 bp, Artificial sequence
  Synthesized
cgctttcctggagcaaatataa

SEQ ID NO: 100 - DNA, 22 bp, Artificial sequence
  Synthesized
ttatatttgctccaggaaagct

SEQ ID NO: 101 - DNA, 22 bp, Artificial sequence
  Synthesized
cggagcaaatataattggtaat

SEQ ID NO: 102 - DNA, 22 bp, Artificial sequence
  Synthesized
attaccaattatatttgctcca

SEQ ID NO: 103 - DNA, 22 bp, Artificial sequence
  Synthesized
cgctcctgatctgattattaat

SEQ ID NO: 104 - DNA, 22 bp, Artificial sequence
  Synthesized
attaataatcagatcaggagca

SEQ ID NO: 105 - DNA, 22 bp, Artificial sequence
  Synthesized
accaagagctatttgatgaaat

SEQ ID NO: 106 - DNA, 22 bp, Artificial sequence
  Synthesized
atttcatcaaatagctcttggc

SEQ ID NO: 107 - DNA, 22 bp, Artificial sequence
  Synthesized
acagctttacatgcaatttatt

SEQ ID NO: 108 - DNA, 22 bp, Artificial sequence
  Synthesized
aataaattgcatgtaaagctgc

SEQ ID NO: 109 - DNA, 324 bp, Artificial sequence
  Synthesized
ctgtttgaatgaggcttcagtactttacagaatcgttgcctgcacatcttggaaacacttgctgggattacttcgacttcttaacccaacagaaggctcgagaaggtatattgctgttgacagtgagcgaagatgtgatggacttctataatagtgaagccacagatgtattatagaagtccatcacatctctgcctactgcctcggacttcaaggggctagaattcgagcaattatcttgtttactaaaactgaataccttgctatctctttgatacatttttacaaagctgaattaaaatggtataaattaaatcactttgc

SEQ ID NO: 110 - DNA, 324 bp, Artificial sequence
  Synthesized
ctgtttgaatgaggcttcagtactttacagaatcgttgcctgcacatcttggaaacacttgctgggattacttcgacttcttaacccaacagaaggctcgagaaggtatattgctgttgacagtgagcgaaccaacggtggcaatgtgaaatagtgaagccacagatgtatttcacattgccaccgttggtgtgcctactgcctcggacttcaaggggctagaattcgagcaattatcttgtttactaaaactgaataccttgctatctctttgatacatttttacaaagctgaattaaaatggtataaattaaatcactttgc

SEQ ID NO: 111 - DNA, 324 bp, Artificial sequence
  Synthesized
ctgtttgaatgaggcttcagtactttacagaatcgttgcctgcacatcttggaaacacttgctgggattacttcgacttcttaacccaacagaaggctcgagaaggtatattgctgttgacagtgagcgaggtggcaatgtgaaattgtattagtgaagccacagatgtaatacaatttcacattgccaccgtgcctactgcctcggacttcaaggggctagaattcgagcaattatcttgtttactaaaactgaataccttgctatctctttgatacatttttacaaagctgaattaaaatggtataaattaaatcactttgc

SEQ ID NO: 112 - DNA, 324 bp, Artificial sequence
  Synthesized
ctgtttgaatgaggcttcagtactttacagaatcgttgcctgcacatcttggaaacacttgctgggattacttcgacttcttaacccaacagaaggctcgagaaggtatattgctgttgacagtgagcgagcaagctttcctggagcaaattagtgaagccacagatgtaatttgctccaggaaagcttgcctgcctactgcctcggacttcaaggggctagaattcgagcaattatcttgtttactaaaactgaataccttgctatctctttgatacatttttacaaagctgaattaaaatggtataaattaaatcactttgc

SEQ ID NO: 113 - DNA, 324 bp, Artificial sequence
  Synthesized
ctgtttgaatgaggcttcagtactttacagaatcgttgcctgcacatcttggaaacacttgctgggattacttcgacttcttaacccaacagaaggctcgagaaggtatattgctgttgacagtgagcgcgctttcctggagcaaatataatagtgaagccacagatgtattatatttgctccaggaaagcttgcctactgcctcggacttcaaggggctagaattcgagcaattatcttgtttactaaaactgaataccttgctatctctttgatacatttttacaaagctgaattaaaatggtataaattaaatcactttgc

SEQ ID NO: 114 - DNA, 324 bp, Artificial sequence
  Synthesized
ctgtttgaatgaggcttcagtactttacagaatcgttgcctgcacatcttggaaacacttgctgggattacttcgacttcttaacccaacagaaggctcgagaaggtatattgctgttgacagtgagcgcggagcaaatataattggtaattagtgaagccacagatgtaattaccaattatatttgctccatgcctactgcctcggacttcaaggggctagaattcgagcaattatcttgtttactaaaactgaataccttgctatctctttgatacatttttacaaagctgaattaaaatggtataaattaaatcactttgc

SEQ ID NO: 115 - DNA, 324 bp, Artificial sequence
  Synthesized
ctgtttgaatgaggcttcagtactttacagaatcgttgcctgcacatcttggaaacacttgctgggattacttcgacttcttaacccaacagaaggctcgagaaggtatattgctgttgacagtgagcgcgctcctgatctgattattaattagtgaagccacagatgtaattaataatcagatcaggagcatgcctactgcctcggacttcaaggggctagaattcgagcaattatcttgtttactaaaactgaataccttgctatctctttgatacatttttacaaagctgaattaaaatggtataaattaaatcactttgc

SEQ ID NO: 116 - DNA, 324 bp, Artificial sequence
  Synthesized
ctgtttgaatgaggcttcagtactttacagaatcgttgcctgcacatcttggaaacacttgctgggattacttcgacttcttaacccaacagaaggctcgagaaggtatattgctgttgacagtgagcgaccaagagctatttgatgaaattagtgaagccacagatgtaatttcatcaaatagctcttggctgcctactgcctcggacttcaaggggctagaattcgagcaattatcttgtttactaaaactgaataccttgctatctctttgatacatttttacaaagctgaattaaaatggtataaattaaatcactttgc

SEQ ID NO: 117 - DNA, 324 bp, Artificial sequence
  Synthesized
ctgtttgaatgaggcttcagtactttacagaatcgttgcctgcacatcttggaaacacttgctgggattacttcgacttcttaacccaacagaaggctcgagaaggtatattgctgttgacagtgagcgacagctttacatgcaatttatttagtgaagccacagatgtaaataaattgcatgtaaagctgctgcctactgcctcggacttcaaggggctagaattcgagcaattatcttgtttactaaaactgaataccttgctatctctttgatacatttttacaaagctgaattaaaatggtataaattaaatcactttgc

SEQ ID NO: 118 - protein, 182 aa, Homo sapiens
GSHSLKYFHTSVSRPGRGEPRFISVGYVDDTQFVRFDNDAASPRMVPRAPWMEQEGSEYWDRETRSARDTAQIFRVNLRTLRGYYNQSEAGSHTLQWMHGCELGPDGRFLRGYEQFAYDGKDYLTLNEDLRSWTAVDTAAQISEQKSNDASEAEHQRAYLEDTCVEWLHKYLEKGKETLLHL

SEQ ID NO: 119 - protein, 99 aa, Homo sapiens [sequence omitted]

SEQ ID NO: 120 - protein, 9 aa, Homo sapiens
VMAPRTLFL

SEQ ID NO: 121 - DNA, 15 bp, Artificial sequence
  Synthesized
ggggsggggsggggs

SEQ ID NO: 122 - DNA, 20 bp, Artificial sequence
  Synthesized
ggggsggggsggggsggggs

SEQ ID NO: 123 - protein, 163 aa, Chlamydomonas reinhardtii
MNTKYNKEFLLYLAGFVDGDGSIIAQIKPNQSYKFKHQLSLAFQVTQKTQRRWFLDKLVDEIGVGYVRDRGSVSDYILSEIKPLHNFLTQLQPFLKLKQKQANLVLKIIWRLPSAKESPDKFLEVCTWVDQIAALNDSKTRKTTSETVRAVLDSLSEKKKSSP